European Patent Specification EP 3 282 014 B1, published September 6, 2023. Title: Cancer Specific Anti-Podocalyxin Antibody and Manufacturing Method Thereof. Applicant: TOHOKU UNIVERSITY. The sequence listing filed with the application follows.

SEQUENCE LISTING (41 sequences)

SEQ ID NO: 1 - protein, 558 aa, Homo sapiens
MRCALALSALLLLLSTPPLLPSSPSPSPSPSQNATQTTTDSSNKTAPTPASSVTIMATDTAQQSTVPTSKANEILASVKATTLGVSSDSPGTTTLAQQVSGPVNTTVARGGGSGNPTTTIESPKSTKSADTTTVATSTATAKPNTTSSQNGAEDTTNSGGKSSHSVTTDLTSTKAEHLTTPHPTSPLSPRQPTSTHPVATPTSSGHDHLMKISSSSSTVAIPGYTFTSPGMTTTLLETVFHHVSQAGLELLTSGDLPTLASQSAGITASSVISQRTQQTSSQMPASSTAPSSQETVQPTSPATALRTPTLPETMSSSPTAASTTHRYPKTPSPTVAHESNWAKCEDLETQTQSEKQLVLNLTGNTLCAGGASDEKLISLICRAVKATFNPAQDKCGIRLASVPGSQTVVVKEITIHTKLPAKDVYERLKDKWDELKEAGVSDMKLGDQGPPEEAEDRFSMPLIITIVCMASFLLLVAALYGCCHQRLSQRKDQQRLTEELQTVENGYHDNPTLEVMETSSEMQEKKVVSLNGELGDSWIVPLDNLTKDDLDEEEDTHL

SEQ ID NO: 2 - protein, 10 aa, Artificial
  PcMab-6 heavy chain CDR1.
GFNFNTNAMN

SEQ ID NO: 3 - protein, 19 aa, Artificial
  PcMab-6 heavy chain CDR2.
LIRSKSNNYATYYADSVKD

SEQ ID NO: 4 - protein, 5 aa, Artificial
  PcMab-6 heavy chain CDR3.
GYGSY

SEQ ID NO: 5 - protein, 11 aa, Artificial
  PcMab-6 light chain CDR1.
KASQSVNNDVA

SEQ ID NO: 6 - protein, 7 aa, Artificial
  PcMab-6 light chain CDR2.
FASNRYT

SEQ ID NO: 7 - protein, 9 aa, Artificial
  PcMab-6 light chain CDR3.
QLDYNSTWT

SEQ ID NO: 8 - protein, 234 aa, Artificial
  PcMab-6 light chain CDR1.
MKSQTQVFVFLLLCVSGAHGSIVMTQTPKFLLVSAGDRVTITCKASQSVNNDVAWYQQKPGQSPKLLIFFASNRYTGVPDRFTGSGYGTDFTFTISNVQAEDLAVYFCQLDYNSTWTFGGGTKLEIKRADAAPTVSIFPPSSEQLTSGGASVVCFLNNFYPKDINVKWKIDGSERQNGVLNSWTDQDSKDSTYSMSSTLTLTKDEYERHNSYTCEATHKTSTSPIVKSFNRNEC

SEQ ID NO: 9 - DNA, 705 bp, Artificial
  PcMab-6 light chain.
atgaagtcacagacccaggtcttcgtatttctactgctctgtgtgtctggtgctcatgggagtattgtgatgacccagactcccaaattcctgcttgtatcagcaggagacagggttaccataacctgcaaggccagtcagagtgtgaataatgatgtagcttggtaccaacagaagccagggcagtctcctaaactgctgatattctttgcatccaatcgctacactggagtccctgatcgcttcactggcagtggatatgggacggatttcactttcaccatcagcaatgtacaggctgaagacctggcagtttatttctgtcagctggattataactctacgtggacgttcggtggaggcaccaagctggaaatcaaacgggctgatgctgcaccaactgtatccatcttcccaccatccagtgagcagttaacatctggaggtgcctcagtcgtgtgcttcttgaacaacttctaccccaaagacatcaatgtcaagtggaagattgatggcagtgaacgacaaaatggcgtcctgaacagttggactgatcaggacagcaaagacagcacctacagcatgagcagcaccctcacgttgaccaaggacgagtatgaacgacataacagctatacctgtgaggccactcacaagacatcaacttcacccattgtcaagagcttcaacaggaatgagtgttag

SEQ ID NO: 10 - protein, 459 aa, Artificial
  PcMab-6 heavy chain.
MLLGLKWVFFVVFYQGVHCEVQLVETGGGLVQPKGSLKLSCAASGFNFNTNAMNWVRQAPGKGLEWVALIRSKSNNYATYYADSVKDRFTISRDDEQSMLHLQMNNLKTEDTAIYFCVKGYGSYWGQGTTLTVSSAKTTPPSVYPLAPGSAAQTNSMVTLGCLVKGYFPEPVTVTWNSGSLSSGVHTFPAVLQSDLYTLSSSVTVPSSTWPSETVTCNVAHPASSTKVDKKIVPRDCGCKPCICTVPEVSSVFIFPPKPKDVLTITLTPKVTCVVVDISKDDPEVQFSWFVDDVEVHTAQTQPREEQFNSTFRSVSELPIMHQDWLNGKEFKCRVNSAAFPAPIEKTISKTKGRPKAPQVYTIPPPKEQMAKDKVSLTCMITDFFPEDITVEWQWNGQPAENYKNTQPIMDTDGSYFVYSKLNVQKSNWEAGNTFTCSVLHEGLHNHHTEKSLSHSPGK

SEQ ID NO: 11 - DNA, 1380 bp, Artificial
  PcMab-6 heavy chain.
atgctgttggggctgaagtgggttttctttgttgttttttatcaaggtgtacattgtgaggtgcagcttgttgagactggtggaggattggtgcagcctaaagggtcattgaaactctcatgtgcagcctctggattcaacttcaataccaatgccatgaactgggtccgccaggctccaggaaagggtttggaatgggttgctctcataagaagtaaaagtaataattatgcaacatattatgccgattcagtgaaagacaggttcaccatttccagagatgatgaacaaagcatgctccatctgcaaatgaacaacttgaaaactgaggacacagccatttatttctgtgtgaagggctacggtagttactggggccaaggcaccactctcacagtctcctcagccaaaacgacacccccatctgtctatccactggcccctggatctgctgcccaaactaactccatggtgaccctgggatgcctggtcaagggctatttccctgagccagtgacagtgacctggaactctggatccctgtccagcggtgtgcacaccttcccagctgtcctgcagtctgacctctacactctgagcagctcagtgactgtcccctccagcacctggcccagcgagaccgtcacctgcaacgttgcccacccggccagcagcaccaaggtggacaagaaaattgtgcccagggattgtggttgtaagccttgcatatgtacagtcccagaagtatcatctgtcttcatcttccccccaaagcccaaggatgtgctcaccattactctgactcctaaggtcacgtgtgttgtggtagacatcagcaaggatgatcccgaggtccagttcagctggtttgtagatgatgtggaggtgcacacagctcagacgcaaccccgggaggagcagttcaacagcactttccgctcagtcagtgaacttcccatcatgcaccaggactggctcaatggcaaggagttcaaatgcagggtcaacagtgcagctttccctgcccccatcgagaaaaccatctccaaaaccaaaggcagaccgaaggctccacaggtgtacaccattccacctcccaaggagcagatggccaaggataaagtcagtctgacctgcatgataacagacttcttccctgaagacattactgtggagtggcagtggaatgggcagccagcggagaactacaagaacactcagcccatcatggacacagatggctcttacttcgtctacagcaagctcaatgtgcagaagagcaactgggaggcaggaaatactttcacctgctctgtgttacatgagggcctgcacaaccaccatactgagaagagcctctcccactctcctggtaaatga

SEQ ID NO: 12 - DNA, 30 bp, Artificial
  Primer HindIII-PcMab6HF1atg.
gctaagcttaacatgctgttggggctgaag

SEQ ID NO: 13 - DNA, 30 bp, Artificial
  Primer mIgG1terNotI.
ggcggccgctcatttaccaggagagtggga

SEQ ID NO: 14 - DNA, 34 bp, Artificial
  Primer InF.HindIII-Pc47H.
cggtatcgataagcttaacatggaaaggcactgg

SEQ ID NO: 15 - DNA, 34 bp, Artificial
  Primer InF.Pc47HterNotI.
tctagagtcgcggccgctcatttaccaggagagt

SEQ ID NO: 16 - DNA, 30 bp, Artificial
  Primer HindIII-PcMab6L.F1atg.
gcgaagcttaagatgaagtcacagacccag

SEQ ID NO: 17 - DNA, 30 bp, Artificial
  Primer mIgCKterNotI.
ggcggccgcctaacactcattcctgttgaa

SEQ ID NO: 18 - DNA, 36 bp, Artificial
  Primer InF.HindIII-Pc47L.
cggtatcgataagcttaaaatggattttcaggtgca

SEQ ID NO: 19 - DNA, 34 bp, Artificial
  Primer InF.mIgCKterNotI.
tctagagtcgcggccgcctaacactcattcctgt

SEQ ID NO: 20 - protein, 237 aa, Artificial
  PcMab-47 light chain.
MDFQVQIFSFLLISASVIMSRGQIVLTQSPAIMSASLGERVTMYCTASSSVSSSYLHWYQQKPGSSPKLWIYGTSNLASGVPARFSGSGSGTSYSLTISSMEAEDAATYYCHQYHRPPLTFGAGTKLELKRADAAPTVSIFPPSSEQLTSGGASVVCFLNNFYPKDINVKWKIDGSERQNGVLNSWTDQDSKDSTYSMSSTLTLTKDEYERHNSYTCEATHKTSTSPIVKSFNRNEC

SEQ ID NO: 21 - DNA, 714 bp, Artificial
  PcMab-47 light chain.
atggattttcaggtgcagattttcagcttcctgctaatcagtgcctcagtcataatgtccagaggacaaattgttctcacccagtctccagcaatcatgtctgcatctctaggggaacgggtcaccatgtactgcactgccagctcaagtgtaagttccagttacttgcactggtaccagcagaagccaggatcctcccccaaactctggatttatggcacatccaacctggcttctggagtcccagctcgcttcagtggcagtgggtctgggacctcttactctctcacaatcagcagcatggaggctgaagatgctgccacttattactgccaccaatatcatcgtcccccgctcacgttcggtgctgggaccaagctggagctgaaacgggctgatgctgcaccaactgtatccatcttcccaccatccagtgagcagttaacatctggaggtgcctcagtcgtgtgcttcttgaacaacttctaccccaaagacatcaatgtcaagtggaagattgatggcagtgaacgacaaaatggcgtcctgaacagttggactgatcaggacagcaaagacagcacctacagcatgagcagcaccctcacgttgaccaaggacgagtatgaacgacataacagctatacctgtgaggccactcacaagacatcaacttcacccattgtcaagagcttcaacaggaatgagtgttag

SEQ ID NO: 22 - protein, 458 aa, Artificial
  PcMab-47 heavy chain.
MERHWIFLFLLSVTAGVHSQVQLQQSAAELARPGASVKMSCKASGYTFTNYTIHWVKQRPGQGLEWIGFINPTSGYSDFNQKFKAKTTLTADKSSSTAHMQLTSLTSEDSAVYYCARLFAPAYWGQGTLVTVSAAKTTPPSVYPLAPGSAAQTNSMVTLGCLVKGYFPEPVTVTWNSGSLSSGVHTFPAVLQSDLYTLSSSVTVPSSTWPSETVTCNVAHPASSTKVDKKIVPRDCGCKPCICTVPEVSSVFIFPPKPKDVLTITLTPKVTCVVVDISKDDPEVQFSWFVDDVEVHTAQTQPREEQFNSTFRSVSELPIMHQDWLNGKEFKCRVNSAAFPAPIEKTISKTKGRPKAPQVYTIPPPKEQMAKDKVSLTCMITDFFPEDITVEWQWNGQPAENYKNTQPIMDTDGSYFVYSKLNVQKSNWEAGNTFTCSVLHEGLHNHHTEKSLSHSPGK

SEQ ID NO: 23 - DNA, 1377 bp, Artificial
  PcMab-47 heavy chain.
atggaaaggcactggatctttctcttcctgttgtcagtaactgcaggtgtccactcccaggtccagctgcagcagtctgcagctgaactggcaagacctggggcctcagtgaagatgtcctgcaaggcttctggctacacctttactaactacacgatacactgggtaaaacagaggcctggacagggtctggaatggattggattcattaatcctaccagtggatattctgacttcaatcagaagttcaaggccaagaccacattgactgcggacaaatcctccagcacagcccacatgcaactgaccagcctgacatctgaggactctgcggtctattactgtgcaagactcttcgctcctgcttactggggccaagggactctggtcactgtctctgcagccaaaacgacacccccatctgtctatccactggcccctggatctgctgcccaaactaactccatggtgaccctgggatgcctggtcaagggctatttccctgagccagtgacagtgacctggaactctggatccctgtccagcggtgtgcacaccttcccagctgtcctgcagtctgacctctacactctgagcagctcagtgactgtcccctccagcacctggcccagcgagaccgtcacctgcaacgttgcccacccggccagcagcaccaaggtggacaagaaaattgtgcccagggattgtggttgtaagccttgcatatgtacagtcccagaagtatcatctgtcttcatcttccccccaaagcccaaggatgtgctcaccattactctgactcctaaggtcacgtgtgttgtggtagacatcagcaaggatgatcccgaggtccagttcagctggtttgtagatgatgtggaggtgcacacagctcagacgcaaccccgggaggagcagttcaacagcactttccgctcagtcagtgaacttcccatcatgcaccaggactggctcaatggcaaggagttcaaatgcagggtcaacagtgcagctttccctgcccccatcgagaaaaccatctccaaaaccaaaggcagaccgaaggctccacaggtgtacaccattccacctcccaaggagcagatggccaaggataaagtcagtctgacctgcatgataacagacttcttccctgaagacattactgtggagtggcagtggaatgggcagccagcggagaactacaagaacactcagcccatcatggacacagatggctcttacttcgtctacagcaagctcaatgtgcagaagagcaactgggaggcaggaaatactttcacctgctctgtgttacatgagggcctgcacaaccaccatactgagaagagcctctcccactctcctggtaaatga

SEQ ID NO: 24 - protein, 10 aa, Artificial
  PcMab-47 heavy chain CDR1.
GYTFTNYTIH

SEQ ID NO: 25 - protein, 17 aa, Artificial
  PcMab-47 heavy chain CDR2.
FINPTSGYSDFNQKFKA

SEQ ID NO: 26 - protein, 6 aa, Artificial
  PcMab-47 heavy chain CDR3.
LFAPAY

SEQ ID NO: 27 - protein, 12 aa, Artificial
  PcMab-47 light chain CDR1.
TASSSVSSSYLH

SEQ ID NO: 28 - protein, 7 aa, Artificial
  PcMab-47 light chain CDR2.
GTSNLAS

SEQ ID NO: 29 - protein, 9 aa, Artificial
  PcMab-47 light chain CDR3.
HQYHRPPLT

SEQ ID NO: 30 - DNA, 30 bp, Artificial
  Primer PcMab6VHR-BamHI.
gccggatcctgaggagactgtgagagtggt

SEQ ID NO: 31 - DNA, 33 bp, Artificial
  Primer InFr.PcMab47VHR-BamHI.
ggcccttggtggatcctgcagagacagtgacca

SEQ ID NO: 32 - DNA, 30 bp, Artificial
  Primer PcMab6LVL-BamHI.
gccggatccccgtttgatttccagcttggt

SEQ ID NO: 33 - DNA, 33 bp, Artificial
  Primer InF.PcMab47LVL-SpeI.
cagccacagtactagtccgtttcagctccagct

SEQ ID NO: 34 - protein, 465 aa, Artificial
  chPcMab-6 heavy chain.
MLLGLKWVFFVVFYQGVHCEVQLVETGGGLVQPKGSLKLSCAASGFNFNTNAMNWVRQAPGKGLEWVALIRSKSNNYATYYADSVKDRFTISRDDEQSMLHLQMNNLKTEDTAIYFCVKGYGSYWGQGTTLTVSSGSTKGPSVFPLAPCSRSTSESTAALGCLVKDYFPEPVTVSWNSGALTSGVHTFPAVLQSSGLYSLSSVVTVPSSNFGTQTYTCNVDHKPSNTKVDKTVEPKSCDKTHTCPPCPAPELLGGPSVFLFPPKPKDTLMISRTPEVTCVVVDVSHEDPEVQFNWYVDGVEVHNAKTKPREEQYNSTYRVVSVLTVLHQDWLNGKEYKCKVSNKALPAPIEKTISKAKGQPREPQVYTLPPSRDELTKNQVSLTCLVKGFYPSDIAVEWESNGQPENNYKTTPPVLDSDGSFFLYSKLTVDKSRWQQGNVFSCSVMHEALHNHYTQKSLSLSPGK

SEQ ID NO: 35 - DNA, 1398 bp, Artificial
  chPcMab-6 heavy chain.
atgctgttggggctgaagtgggttttctttgttgttttttatcaaggtgtacattgtgaggtgcagcttgttgagactggtggaggattggtgcagcctaaagggtcattgaaactctcatgtgcagcctctggattcaacttcaataccaatgccatgaactgggtccgccaggctccaggaaagggtttggaatgggttgctctcataagaagtaaaagtaataattatgcaacatattatgccgattcagtgaaagacaggttcaccatttccagagatgatgaacaaagcatgctccatctgcaaatgaacaacttgaaaactgaggacacagccatttatttctgtgtgaagggctacggtagttactggggccaaggcaccactctcacagtctcctcaggatccaccaagggcccatcggtcttccccctggcgccctgctccaggagcacctccgagagcacagcggccctgggctgcctggtcaaggactacttccccgaaccggtgacggtgtcgtggaactcaggcgctctgaccagcggcgtgcacaccttcccagctgtcctacagtcctcaggactctactccctcagcagcgtggtgaccgtgccctccagcaacttcggcacccagacctacacctgcaacgtagatcacaagcccagcaacaccaaggtggacaagacagttgagcccaaatcttgtgacaaaactcacacatgcccaccgtgcccagcacctgaactcctggggggaccgtcagtcttcctcttccccccaaaacccaaggacaccctcatgatctcccggacccctgaggtcacgtgcgtggtggtggacgtgagccacgaagaccccgaggtccagttcaactggtacgtggacggcgtggaggtgcataatgccaagacaaagccgcgggaggagcagtacaacagcacgtaccgtgtggtcagcgtcctcaccgtcctgcaccaggactggctgaatggcaaggagtacaaatgcaaggtctccaacaaagccctcccagcccccatcgagaaaaccatctccaaagccaaagggcagccccgagaaccacaggtgtacaccctgcccccatcccgggatgagctgaccaagaaccaggtcagcctgacctgcctggtcaaaggcttctatcccagcgacatcgccgtggagtgggagagcaatgggcagccggagaacaactacaagaccacgcctcccgtgctggactccgacggctccttcttcctttacagcaagctcaccgtggacaagagcaggtggcagcaggggaacgtcttctcatgctccgtgatgcatgaggctctgcacaaccactacacgcagaagagcctctccctgtctccgggtaaatga

SEQ ID NO: 36 - protein, 236 aa, Artificial
  chPcMab-6 light chain.
MKSQTQVFVFLLLCVSGAHGSIVMTQTPKFLLVSAGDRVTITCKASQSVNNDVAWYQQKPGQSPKLLIFFASNRYTGVPDRFTGSGYGTDFTFTISNVQAEDLAVYFCQLDYNSTWTFGGGTKLEIKRGSTVAAPSVFIFPPSDEQLKSGTASVVCLLNNFYPREAKVQWKVDNALQSGNSQESVTEQDSKDSTYSLSSTLTLSKADYEKHKVYACEVTHQGLSSPVTKSFNRGEC

SEQ ID NO: 37 - DNA, 711 bp, Artificial
  chPcMab-6 light chain.
atgaagtcacagacccaggtcttcgtatttctactgctctgtgtgtctggtgctcatgggagtattgtgatgacccagactcccaaattcctgcttgtatcagcaggagacagggttaccataacctgcaaggccagtcagagtgtgaataatgatgtagcttggtaccaacagaagccagggcagtctcctaaactgctgatattctttgcatccaatcgctacactggagtccctgatcgcttcactggcagtggatatgggacggatttcactttcaccatcagcaatgtacaggctgaagacctggcagtttatttctgtcagctggattataactctacgtggacgttcggtggaggcaccaagctggaaatcaaacggggatccactgtggctgcaccatctgtcttcatcttcccgccatctgatgagcagttgaaatctggaactgcctctgttgtgtgcctgctgaataacttctatcccagagaggccaaagtacagtggaaggtggataacgccctccaatcgggtaactcccaggagagtgtcacagagcaggacagcaaggacagcacctacagcctcagcagcaccctgacgctgagcaaagcagactacgagaaacacaaagtctacgcctgcgaagtcacccatcagggcctgagctcgcccgtcacaaagagcttcaacaggggagagtgttag

SEQ ID NO: 38 - protein, 464 aa, Artificial
  chPcMab-47 heavy chain.
MERHWIFLFLLSVTAGVHSQVQLQQSAAELARPGASVKMSCKASGYTFTNYTIHWVKQRPGQGLEWIGFINPTSGYSDFNQKFKAKTTLTADKSSSTAHMQLTSLTSEDSAVYYCARLFAPAYWGQGTLVTVSAGSTKGPSVFPLAPCSRSTSESTAALGCLVKDYFPEPVTVSWNSGALTSGVHTFPAVLQSSGLYSLSSVVTVPSSNFGTQTYTCNVDHKPSNTKVDKTVEPKSCDKTHTCPPCPAPELLGGPSVFLFPPKPKDTLMISRTPEVTCVVVDVSHEDPEVQFNWYVDGVEVHNAKTKPREEQYNSTYRVVSVLTVLHQDWLNGKEYKCKVSNKALPAPIEKTISKAKGQPREPQVYTLPPSRDELTKNQVSLTCLVKGFYPSDIAVEWESNGQPENNYKTTPPVLDSDGSFFLYSKLTVDKSRWQQGNVFSCSVMHEALHNHYTQKSLSLSPGK

SEQ ID NO: 39 - DNA, 1395 bp, Artificial
  chPcMab-47 heavy chain.
atggaaaggcactggatctttctcttcctgttgtcagtaactgcaggtgtccactcccaggtccagctgcagcagtctgcagctgaactggcaagacctggggcctcagtgaagatgtcctgcaaggcttctggctacacctttactaactacacgatacactgggtaaaacagaggcctggacagggtctggaatggattggattcattaatcctaccagtggatattctgacttcaatcagaagttcaaggccaagaccacattgactgcggacaaatcctccagcacagcccacatgcaactgaccagcctgacatctgaggactctgcggtctattactgtgcaagactcttcgctcctgcttactggggccaagggactctggtcactgtctctgcaggatccaccaagggcccatcggtcttccccctggcgccctgctccaggagcacctccgagagcacagcggccctgggctgcctggtcaaggactacttccccgaaccggtgacggtgtcgtggaactcaggcgctctgaccagcggcgtgcacaccttcccagctgtcctacagtcctcaggactctactccctcagcagcgtggtgaccgtgccctccagcaacttcggcacccagacctacacctgcaacgtagatcacaagcccagcaacaccaaggtggacaagacagttgagcccaaatcttgtgacaaaactcacacatgcccaccgtgcccagcacctgaactcctggggggaccgtcagtcttcctcttccccccaaaacccaaggacaccctcatgatctcccggacccctgaggtcacgtgcgtggtggtggacgtgagccacgaagaccccgaggtccagttcaactggtacgtggacggcgtggaggtgcataatgccaagacaaagccgcgggaggagcagtacaacagcacgtaccgtgtggtcagcgtcctcaccgtcctgcaccaggactggctgaatggcaaggagtacaaatgcaaggtctccaacaaagccctcccagcccccatcgagaaaaccatctccaaagccaaagggcagccccgagaaccacaggtgtacaccctgcccccatcccgggatgagctgaccaagaaccaggtcagcctgacctgcctggtcaaaggcttctatcccagcgacatcgccgtggagtgggagagcaatgggcagccggagaacaactacaagaccacgcctcccgtgctggactccgacggctccttcttcctttacagcaagctcaccgtggacaagagcaggtggcagcaggggaacgtcttctcatgctccgtgatgcatgaggctctgcacaaccactacacgcagaagagcctctccctgtctccgggtaaatga

SEQ ID NO: 40 - protein, 239 aa, Artificial
  chPcMab-47 light chain.
MDFQVQIFSFLLISASVIMSRGQIVLTQSPAIMSASLGERVTMYCTASSSVSSSYLHWYQQKPGSSPKLWIYGTSNLASGVPARFSGSGSGTSYSLTISSMEAEDAATYYCHQYHRPPLTFGAGTKLELKRTSTVAAPSVFIFPPSDEQLKSGTASVVCLLNNFYPREAKVQWKVDNALQSGNSQESVTEQDSKDSTYSLSSTLTLSKADYEKHKVYACEVTHQGLSSPVTKSFNRGEC

SEQ ID NO: 41 - DNA, 720 bp, Artificial
  chPcMab-47 light chain.
atggattttcaggtgcagattttcagcttcctgctaatcagtgcctcagtcataatgtccagaggacaaattgttctcacccagtctccagcaatcatgtctgcatctctaggggaacgggtcaccatgtactgcactgccagctcaagtgtaagttccagttacttgcactggtaccagcagaagccaggatcctcccccaaactctggatttatggcacatccaacctggcttctggagtcccagctcgcttcagtggcagtgggtctgggacctcttactctctcacaatcagcagcatggaggctgaagatgctgccacttattactgccaccaatatcatcgtcccccgctcacgttcggtgctgggaccaagctggagctgaaacggactagtactgtggctgcaccatctgtcttcatcttcccgccatctgatgagcagttgaaatctggaactgcctctgttgtgtgcctgctgaataacttctatcccagagaggccaaagtacagtggaaggtggataacgccctccaatcgggtaactcccaggagagtgtcacagagcaggacagcaaggacagcacctacagcctcagcagcaccctgacgctgagcaaagcagactacgagaaacacaaagtctacgcctgcgaagtcacccatcagggcctgagctcgcccgtcacaaagagcttcaacaggggagagtgttag